European Patent Application EP 4 578 955 A1, published July 2, 2025. Title: METHOD FOR SYNTHESIZING PURINE NUCLEOSIDE THROUGH ENZYMATIC CATALYSIS AND COMPOSITION. Applicant: Asymchem Laboratories(Tianjin) Co.,Ltd. The sequence listing filed with the application follows.

SEQUENCE LISTING (6 sequences)

SEQ ID NO: 1 - protein, 423 aa, Thermus thermophilus
MNPVAFIREKREGKKHRREDLEAFLLGYLRDEVPDYQVSAWLMAAFLRGLDPEETLWLTETMARSGKVLDLSGLPHPVDKHSSGGVGDKVSLVVGPILAASGCTFAKMSGRGLAHTGGTIDKLESVPGWRGEMTEAEFLERARRVGLVIAAQSPDLAPLDGKLYALRDVTATVESVPLIASSIMSKKLAAGARSIVLDVKVGRGAFMKTLEEARLLAKTMVAIGQGAGRRVRALLTSMEAPLGRAVGNAIEVREAIEALKGEGPGDLLEVALALAEEALRLEGLDPALARKALEGGAALEKFRAFLEAQGGDPRAVEDFSLLPLAEEHPLRAEREGVVREVDAYKVGLAVLALGGGRKRKGEPIDHGVGVYLLKKPGDRVERGEALALVYHRRRGLEEALGHLREAYALGEEAHPAPLVLEAI

SEQ ID NO: 2 - protein, 482 aa, Homo sapiens [sequence omitted]

SEQ ID NO: 3 - protein, 234 aa, Geobacillus stearothermophilus
MSVHIGAKEHEIADKILLPGDPLRAKYIAETFLEGATCYNQVRGMLGFTGTYKGHRISVQGTGMGVPSISIYITELMQSYNVQTLIRVGTCGAIQKDVKVRDVILAMTSSTDSQMNRMTFGGIDYAPTANFDLLKTAYEIGKEKGLQLKVGSVFTADMFYNENAQFEKLARYGVLAVEMETTALYTLAAKFGRKALSVLTVSDHILTGEETTAEERQTTFNEMIEVALETAIRQ

SEQ ID NO: 4 - DNA, 1272 bp, synthetic construct
  source 1..1272: mol_type = other DNA; note = DNA sequence encoding PyNP
atgaacccggtggcgtttattcgcgaaaaacgcgaaggcaagaaacatcgccgcgaggatctggaagcgtttctgctgggctatctgcgcgatgaagtgccggattatcaggtgagcgcgtggctgatggcggcgtttttacgcggcttagatccggaagaaaccctgtggctgaccgaaacgatggcccgcagcggtaaagtgctggatctgagcggtctgccgcatccggttgataaacatagcagcggcggcgtgggcgataaagtgagcttagtggtgggcccgattctggcggcgagcggttgtacctttgcgaaaatgtcgggccgcggcctggcgcataccggtggtaccattgataaactggaaagcgtgccgggctggcgcggcgaaatgaccgaagcagaatttctggaacgcgcccgtcgcgttggtctggttattgcggcgcaaagcccggatttagcgccgttagatggcaaactgtatgcgctgcgcgatgtgaccgcgaccgttgaatcagttccgctgattgcgagcagcattatgagcaagaaactggcggcgggcgcccgtagcattgtgttagatgttaaagtgggccgcggcgcgtttatgaaaaccctggaagaagcgcgtctgctggcgaaaacgatggtggcgattggccagggcgcgggccgtcgtgttcgtgcgttattaaccagcatggaagcgcctctgggtcgtgcggttggcaatgcgattgaagtgcgtgaagcgattgaagcgctgaaaggcgaaggcccgggcgatttattagaagtggcgctggcgttagcggaagaagcgctgcgtttagaaggcttagatccggcgctggcgcgtaaagcgttagaaggtggcgcggcgctggaaaaatttcgcgcgtttctggaagcgcagggcggcgatccgcgtgcagttgaagattttagcctgctgccgctggcggaagaacatccgttacgtgcggaacgcgaaggcgtggttcgcgaagttgatgcgtataaagtgggcctggcggtgctggcgttaggcggtggtcgtaaacgtaaaggtgaaccgattgatcatggcgtgggcgtgtatctgctgaagaaaccgggcgatcgcgtggaacgcggcgaagcgttagcgttagtgtatcatcgccgccgcggcttagaagaagcgctgggtcatttacgcgaagcgtatgcgctgggcgaagaagcgcatccggcgcctctggttttagaagcgatttaa

SEQ ID NO: 5 - DNA, 1449 bp, synthetic construct
  source 1..1449: mol_type = other DNA; note = DNA sequence encoding TP
atggcggcgttaatgacccctggcaccggtgcgcctcctgcgcctggtgattttagcggcgaaggcagccagggcctgccggaccctagccctgaacctaaacaactgccggaactgattcgcatgaaacgcgatggtggccgcctgagcgaagcggatattcgcggttttgtggcggcggtggtgaacggcagcgcacaaggtgcgcaaattggtgcgatgttaatggcgattcgcctgcgcggcatggatctggaagaaaccagcgtgctgacccaggcgctggcgcaaagcggtcagcaactggaatggcctgaagcgtggcgccagcagttagttgataaacatagcaccggcggcgtgggcgataaagtgagcttagttctggcgccggcgctggcggcgtgtggctgtaaagttcctatgattagcggccgtggcctgggccataccggtggtactttagataaactggaaagcattccgggctttaacgtgattcagagcccggaacagatgcaggtgctgctggatcaggcgggctgttgcattgtgggccagagcgaacagctggtgccggcggaagggattctgtatgcggcgcgtgatgtgaccgcgaccgttgatagcttaccgctgattaccgcgagcattctgagcaaaaagctggtggaaggcctgagcgccctggtggtggatgttaaatttggcggcgcggcggtgtttccgaaccaggaacaagcccgcgaactggcgaaaaccctggtgggcgttggcgcgagcctgggtttacgtgttgcggcggcgttaaccgcgatggataaaccgttaggccgctgcgttggccatgcgctggaagtggaagaagcgctgctgtgcatggatggcgcgggccctcctgatttacgcgatctggttacgaccctgggcggcgcgttactgtggttaagcggccatgcgggtacccaggcgcaaggcgcagcgcgtgttgcggcagcgctggatgatggtagcgcgttaggtcgttttgaacgcatgctggcggcgcagggtgtggaccctggtttggcgcgtgcgttatgtagcggcagccctgcggaacgtcgccagttattacctcgcgcccgtgaacaagaagaactgctggcgccggcggatggcaccgttgaattagtgcgtgcgctgccgttagcgctggtgttacatgaactgggcgcgggccgctcacgtgcgggtgaacctttacgtttaggcgttggtgcggaactgctggtggatgttggtcagcgcctgcgccgtggtaccccttggttacgtgttcatcgtgatggtccggcgctgagcggccctcaaagccgtgcgctgcaagaagcgttagttctgagcgatcgtgcgccgtttgcggcgccgagcccttttgcggaattggttttaccgcctcagcaataa

SEQ ID NO: 6 - DNA, 705 bp, synthetic construct
  source 1..705: mol_type = other DNA; note = DNA sequence encoding PNP
atgagcgtgcatattggcgcgaaagaacatgaaattgcggataaaattctgctgccgggcgatccgttacgcgcgaaatatattgcggaaacctttctggaaggcgcgacctgctataaccaggtgcgcggcatgctgggctttaccggcacctataaaggccatcgcattagcgtgcagggcaccggcatgggcgttcctagcatttcaatttatattaccgaactgatgcagagctataacgtgcagaccctgattcgcgtgggcacctgcggtgcgattcaaaaagatgtgaaagtgcgcgatgtgattctggcgatgaccagcagcaccgatagccagatgaaccgcatgacctttggcggcattgattatgcgccgaccgcgaactttgatctgctgaaaaccgcgtatgaaattggcaaagaaaaaggcctgcagctgaaagtgggcagcgtgtttaccgcggatatgttttataacgaaaacgcgcagtttgagaaactggcccgctatggcgtgctggcggttgaaatggaaaccaccgcgctgtataccctggcggcgaaatttggccgcaaagcgctgagcgtgctgaccgtgagcgatcatattctgaccggcgaagaaaccaccgcggaagaacgccagaccacctttaacgaaatgattgaagtggcgctggaaaccgcgattcgccagtaa